European Patent Specification EP 3 572 513 B1, published September 24, 2025. Title: HIPPO AND DYSTROPHIN COMPLEX SIGNALING IN CARDIOMYOCYTE RENEWAL. Applicant: Martin, James F. Yuka, Morikawa Todd, Heallen Ryan Leach, John. Application UNKNOWN. The sequence listing filed with the application follows.

SEQUENCE LISTING (12 sequences)

SEQ ID NO: 1 - DNA, 1161 bp, Mus musculus
atgctgtcccgcaagaaaaccaaaaacgaggtgtctaagccggccgaggtgcagggcaagtacgtgaagaaggagacgtcgcccctgctgcggaatctcatgccttcattcattcggcacggtccaacaattcccagacggactgacctctgtcttccagattcaagtgctactgctttctcagcttctggagatggtgtagtttcaagaaaccagagtttcctgagaactgcaattcaaaggacacctcatgaagtaatgagaagagaaagccacagactgtctgccccttcttaccttgtcaggagcctagcagatgtccctcgagagtgtggctcatcacagtcatttttgacagaagttaactttgctgttgagaatggagactctggctcccgatacttcttctcagataacttttttgatggacagagaaggcggccacttggagatcgtgcacaagaagattacagatattatgaatacaaccatgatctcttccagaggatgccacagagtcaggggaggcacacttcaggtattgggagagtcacggctacatctctagggaatttaactaaccatggatctgaagatttaccccttcctcctggctggtctgtggactggacaatgagagggagaaaatactacatagatcataacacaaataccactcactggagtcatccccttgaacgagaaggacttcctcctggctgggaacgagtagagtcatcagaatttggaacctattacgtggatcacaccaataaaagggctcagtacaggcacccctgtgctccgagtgtacctcggtatgatcagcctccacccatcacgtatcagccacaacaaactgaaagaaatcagtctctcctggtccctgcaaatccctaccatactgcagaaattcctgactggcttcaggtttatgcccgagcccctgtgaaatatgaccacattctgaagtgggagctcttccagctggctgacctggacacgtaccagggaatgctgaagttgctcttcatgaaggaactggagcagattgtgaagttgtacgaggcctacagacaggctcttctcactgagttggaaaaccgcaagcagaggcagcagtggtatgcccagcagcatggcaagacgttcttaagttaa

SEQ ID NO: 2 - DNA, 1155 bp, Sus scrofa
atgctgtcccgaaagaaaaccaaaaatgaagtgtccaagccggccgaggtgcaggggaagtacgtgaagaaggagacgtcgcctctgctgcggaatctcatgccttcattcatccggcacggtcccacaattccaagacgaactgatatctgtcttccagattccagctctaatgccttttcagcttctggagatggaatagtttcaagaaaccagagtttccttagaactccaattcaaagaacacctcatgaaataatgagaagagaaagcaacagattatctgcaccttcttatcttgccaggagtctagcagatgtccctagggaatatggctcttctcagtcatttttaacagaagttaattttgctgttgaaaatggagactctggttcccgatattattattccgataattattttgatggtcagaggaggcgccagcttggagatcgcacacatgaagactatagatattatgactacaaccacgatctcttccaaagagtgccacaaaatcaggggaggcatgcttcaggtattgggagaattgctgctacatctttaggaaatttaacaaaccatggttctgaagatttaccccttcctcctggctggtctgtggactggacaatgagagggaggaaatactatatagatcacaacacaaatacaactcattggagccatcctcttgagcgagaaggacttcctccaggatgggagcgagttgagtcatcagaatttggaacctattatgtagatcacacaaataaaaaggctcaatataggcatccctgtgctcctagcgtacctcgatatgatcaacctcctcctgttacataccagccacagcaaactgaaagaaatcagtcccttctggtacctgcaaatccgtatcatgctgcagaaattcctgactggcttcaggtttatgctcgagcccctgtgaaatatgaccacattctcaagtgggaactcttccagctggctgacctggatacataccagggaatgctgaagttgcttttcatgaaagaactggaacagattgttaaaatgtatgaagcctacagacaggctcttctcacagagttggaaaatcgcaagcagagacaacagtggtatgcccagcaacatggcaagaatttttaa

SEQ ID NO: 3 - DNA, 1152 bp, Homo sapiens
atgctgtcccgaaagaaaaccaaaaacgaagtgtccaagccggccgaggtgcaggggaagtacgtgaagaaggagacgtcgcctctgcttcggaatcttatgccttcattcatccggcatggtccaacaattccaagacgaactgatatctgtcttccagattcaagccctaatgccttttcaacttctggagatgtagtttcaagaaaccagagtttccttagaactccaattcaaagaacacctcatgaaataatgagaagagaaagcaacagattatctgcaccttcttatcttgccagaagtctagcagatgtccctagagagtatggttcttctcagtcatttgtaacggaagttagttttgctgttgaaaatggagactctggttcccgatattattattcagacaatttttttgatggtcagagaaagcggccacttggagatcgtgcacatgaagactacagatattatgaatacaaccatgatctcttccaaagaatgccacagaatcaggggaggcatgcttcaggtattgggagagttgctgctacatctttaggaaatttgactaaccatggttctgaagatttaccccttcctcctggctggtctgtggactggacaatgagagggagaaaatattatatagatcataacacaaatacaactcactggagccatcctcttgagcgagaaggacttcctcctggatgggaacgagttgagtcatccgaatttggaacctattatgtagatcacacaaataagaaggcccaatacaggcatccctgtgctcctagtgtacctcggtatgatcaaccacctcctgtcacataccagccacagcaaactgaaagaaatcagtcccttctggtacctgcaaatccatatcatactgcagaaattcctgactggcttcaggtttacgcacgagcccctgtgaaatatgaccacattctgaagtgggaactcttccagctggctgacctggatacataccagggaatgctaaagttgctcttcatgaaagaattggagcagattgttaaaatgtatgaagcatacagacaagcccttcttacagagttggaaaaccgaaagcagagacagcagtggtatgcccaacaacatggaaaaaatttttga

SEQ ID NO: 4 - DNA, 21 bp, Mus musculus
aagtacgtgaagaaggagacg

SEQ ID NO: 5 - DNA, 21 bp, Mus musculus
aagatttaccccttcctcctg

SEQ ID NO: 6 - DNA, 20 bp, Mus musculus
attcctgactggcttcaggt

SEQ ID NO: 7 - DNA, 21 bp, Sus scrofa
aagtacgtgaagaaggagacg

SEQ ID NO: 8 - DNA, 21 bp, Sus scrofa
aagatttaccccttcctcctg

SEQ ID NO: 9 - DNA, 20 bp, Sus scrofa
attcctgactggcttcaggt

SEQ ID NO: 10 - DNA, 21 bp, Homo sapiens
aagtacgtgaagaaggagacg

SEQ ID NO: 11 - DNA, 21 bp, Homo sapiens
aagatttaccccttcctcctg

SEQ ID NO: 12 - DNA, 20 bp, Homo sapiens
attcctgactggcttcaggt